European Patent Application EP 4 696 772 A1, published February 18, 2026. Title: 적혈구 전구세포 분화 유도용 조성물. Applicant: 한양대학교 산학협력단. The sequence listing filed with the application follows.

SEQUENCE LISTING (20 sequences)

SEQ ID NO: 1 - DNA, 20 bp, synthetic construct
  source 1..20: mol_type = other DNA
ccaacgtgtcagtggtggac

SEQ ID NO: 2 - DNA, 23 bp, synthetic construct
  source 1..23: mol_type = other DNA
cctgcactttttaagagccagtc

SEQ ID NO: 3 - DNA, 20 bp, synthetic construct
  source 1..20: mol_type = other DNA
gaagctcagcgtcctcaaga

SEQ ID NO: 4 - DNA, 19 bp, synthetic construct
  source 1..19: mol_type = other DNA
ctggtcgctgctatgctct

SEQ ID NO: 5 - DNA, 20 bp, synthetic construct
  source 1..20: mol_type = other DNA
ccacagtaaggcaggctgta

SEQ ID NO: 6 - DNA, 20 bp, synthetic construct
  source 1..20: mol_type = other DNA
ggaacaggtcatggtcacag

SEQ ID NO: 7 - DNA, 18 bp, synthetic construct
  source 1..18: mol_type = other DNA
gaagatgctggcgtgaca

SEQ ID NO: 8 - DNA, 18 bp, synthetic construct
  source 1..18: mol_type = other DNA
gctgcctccacctctaag

SEQ ID NO: 9 - DNA, 19 bp, synthetic construct
  source 1..19: mol_type = other DNA
tgaggtggggaccagccgg

SEQ ID NO: 10 - DNA, 20 bp, synthetic construct
  source 1..20: mol_type = other DNA
gtgaccaggacacacagcgg

SEQ ID NO: 11 - DNA, 19 bp, synthetic construct
  source 1..19: mol_type = other DNA
tgaggtggggaccagccgg

SEQ ID NO: 12 - DNA, 20 bp, synthetic construct
  source 1..20: mol_type = other DNA
gtgaccaggacacacagcgg

SEQ ID NO: 13 - DNA, 20 bp, synthetic construct
  source 1..20: mol_type = other DNA
cacacaggatggcttgaaga

SEQ ID NO: 14 - DNA, 20 bp, synthetic construct
  source 1..20: mol_type = other DNA
agggcagaatcatcacgaag

SEQ ID NO: 15 - DNA, 20 bp, synthetic construct
  source 1..20: mol_type = other DNA
cccttgtagggatcctcctc

SEQ ID NO: 16 - DNA, 20 bp, synthetic construct
  source 1..20: mol_type = other DNA
ctcccaaagtgctgggatta

SEQ ID NO: 17 - DNA, 20 bp, synthetic construct
  source 1..20: mol_type = other DNA
catggatgaaggctcagaag

SEQ ID NO: 18 - DNA, 20 bp, synthetic construct
  source 1..20: mol_type = other DNA
tgccagagtcagataccaca

SEQ ID NO: 19 - DNA, 20 bp, synthetic construct
  source 1..20: mol_type = other DNA
ttgaaggagttcagcgttct

SEQ ID NO: 20 - DNA, 20 bp, synthetic construct
  source 1..20: mol_type = other DNA
tgtcacctgctgcctgtaat